European Patent Application EP 4 647 441 A1, published November 12, 2025. Title: TCR MOLECULE TARGETING KRAS G12 MUTATION, AND CELL AND USE THEREOF. Applicant: BEIJING DCTY BIOTECH CO., LTD. The sequence listing filed with the application follows.

SEQUENCE LISTING (17 sequences)

SEQ ID NO: 1 - protein, 275 aa, synthetic construct
METLLGLLILWLQLQWVSSKQEVTQIPAALSVPEGENLVLNCSFTDSAIYNLQWFRQDPGKGLTSLLLIQSSQREQTSGRLNASLDKSSGRSTLYIAASQPGDSATYLCAVNSYSGAGSYQLTFGKGTKLSVIPNIQNPDPAVYQLRDSKSSDKSVCLFTDFDSQTNVSQSKDSDVYITDKTVLDMRSMDFKSNSAVAWSNKSDFACANAFNNSIIPEDTFFPSPESSCDVKLVEKSFETDTNLNFQNLSVIGFRILLLKVAGFNLLMTLRLWSS

SEQ ID NO: 2 - protein, 115 aa, synthetic construct
KQEVTQIPAALSVPEGENLVLNCSFTDSAIYNLQWFRQDPGKGLTSLLLIQSSQREQTSGRLNASLDKSSGRSTLYIAASQPGDSATYLCAVNSYSGAGSYQLTFGKGTKLSVIP

SEQ ID NO: 3 - protein, 6 aa, synthetic construct
DSAIYN

SEQ ID NO: 4 - protein, 7 aa, synthetic construct
IQSSQRE

SEQ ID NO: 5 - protein, 14 aa, synthetic construct
AVNSYSGAGSYQLT

SEQ ID NO: 6 - protein, 309 aa, synthetic construct
MDTWLVCWAIFSLLKAGLTEPEVTQTPSHQVTQMGQEVILRCVPISNHLYFYWYRQILGQKVEFLVSFYNNEISEKSEIFDDQFSVERPDGSNFTLKIRSTKLEDSAMYFCASRGGGEQYFGPGTRLTVTEDLKNVFPPEVAVFEPSEAEISHTQKATLVCLATGFYPDHVELSWWVNGKEVHSGVSTDPQPLKEQPALNDSRYCLSSRLRVSATFWQNPRNHFRCQVQFYGLSENDEWTQDRAKPVTQIVSAEAWGRADCGFTSESYQQGVLSATILYEILLGKATLYAVLVSALVLMAMVKRKDSRG

SEQ ID NO: 7 - protein, 111 aa, synthetic construct
EPEVTQTPSHQVTQMGQEVILRCVPISNHLYFYWYRQILGQKVEFLVSFYNNEISEKSEIFDDQFSVERPDGSNFTLKIRSTKLEDSAMYFCASRGGGEQYFGPGTRLTVT

SEQ ID NO: 8 - protein, 5 aa, synthetic construct
SNHLY

SEQ ID NO: 9 - protein, 6 aa, synthetic construct
FYNNEI

SEQ ID NO: 10 - protein, 9 aa, synthetic construct
ASRGGGEQY

SEQ ID NO: 11 - protein, 10 aa, synthetic construct
VVVGAXGVGK

SEQ ID NO: 12 - protein, 10 aa, synthetic construct
VVVGAVGVGK

SEQ ID NO: 13 - protein, 10 aa, synthetic construct
VVVGADGVGK

SEQ ID NO: 14 - protein, 10 aa, synthetic construct
VVVGASGVGK

SEQ ID NO: 15 - protein, 10 aa, synthetic construct
VVVGAAGVGK

SEQ ID NO: 16 - protein, 10 aa, synthetic construct
VVVGACGVGK

SEQ ID NO: 17 - protein, 10 aa, synthetic construct
VVVGAGGVGK